European Patent Specification EP 3 333 183 B1, published February 22, 2023. Title: TARGETED/IMMUNOMODULATORY FUSION PROTEINS AND METHODS FOR MAKING SAME. Applicant: Biocon Limited. The sequence listing filed with the application follows.

SEQUENCE LISTING (36 sequences)

SEQ ID NO: 1 - protein, 449 aa, Artificial Sequence
  Synthetic construct
EVQLVESGGGLVQPGGSLRLSCAASGFNIKDTYIHWVRQAPGKGLEWVARIYPTNGYTRYADSVKGRFTISADTSKNTAYLQMNSLRAEDTAVYYCSRWGGDGFYAMDYWGQGTLVTVSSASTKGPSVFPLAPSSKSTSGGTAALGCLVKDYFPEPVTVSWNSGALTSGVHTFPAVLQSSGLYSLSSVVTVPSSSLGTQTYICNVNHKPSNTKVDKKVEPKSCDKTHTCPPCPAPELLGGPSVFLFPPKPKDTLMISRTPEVTCVVVDVSHEDPEVKFNWYVDGVEVHNAKTKPREEQYNSTYRVVSVLTVLHQDWLNGKEYKCKVSNKALPAPIEKTISKAKGQPREPQVYTLPPSREEMTKNQVSLTCLVKGFYPSDIAVEWESNGQPENNYKTTPPVLDSDGSFFLYSKLTVDKSRWQQGNVFSCSVMHEALHNHYTQKSLSLSPG

SEQ ID NO: 2 - protein, 214 aa, Artificial Sequence
  Synthetic construct
DIQMTQSPSSLSASVGDRVTITCRASQDVNTAVAWYQQKPGKAPKLLIYSASFLYSGVPSRFSGSRSGTDFTLTISSLQPEDFATYYCQQHYTTPPTFGQGTKVEIKRTVAAPSVFIFPPSDEQLKSGTASVVCLLNNFYPREAKVQWKVDNALQSGNSQESVTEQDSKDSTYSLSSTLTLSKADYEKHKVYACEVTHQGLSSPVTKSFNRGEC

SEQ ID NO: 3 - protein, 15 aa, Artificial Sequence
  Synthetic construct
GGGGSGGGGSGGGGS

SEQ ID NO: 4 - protein, 137 aa, Artificial Sequence
  Synthetic construct
TIPPHVQKSVNNDMIVTDNNGAVKFPQLCKFCDVRFSTCDNQKSCMSNCSITSICEKPQEVCVAVWRKNDENITLETVCHDPKLPYHDFILEDAASPKCIMKEKKKPGETFFMCSCSSDECNDNIIFSEEYNTSNPD

SEQ ID NO: 5 - protein, 448 aa, Artificial Sequence
  Synthetic Construct
QVQLKQSGPGLVQPSQSLSITCTVSGFSLTNYGVHWVRQSPGKGLEWLGVIWSGGNTDYNTPFTSRLSINKDNSKSQVFFKMNSLQSNDTAIYYCARALTYYDYEFAYWGQGTLVTVSAASTKGPSVFPLAPSSKSTSGGTAALGCLVKDYFPEPVTVSWNSGALTSGVHTFPAVLQSSGLYSLSSVVTVPSSSLGTQTYICNVNHKPSNTKVDKRVEPKSCDKTHTCPPCPAPELLGGPSVFLFPPKPKDTLMISRTPEVTCVVVDVSHEDPEVKFNWYVDGVEVHNAKTKPREEQYNSTYRVVSVLTVLHQDWLNGKEYKCKVSNKALPAPIEKTISKAKGQPREPQVYTLPPSRDELTKNQVSLTCLVKGFYPSDIAVEWESNGQPENNYKTTPPVLDSDGSFFLYSKLTVDKSRWQQGNVFSCSVMHEALHNHYTQKSLSLSPG

SEQ ID NO: 6 - protein, 214 aa, Artificial Sequence
  Synthetic construct
DILLTQSPVILSVSPGERVSFSCRASQSIGTNIHWYQQRTNGSPRLLIKYASESISGIPSRFSGSGSGTDFTLSINSVESEDIADYYCQQNNNWPTTFGAGTKLELKRTVAAPSVFIFPPSDEQLKSGTASVVCLLNNFYPREAKVQWKVDNALQSGNSQESVTEQDSKDSTYSLSSTLTLSKADYEKHKVYACEVTHQGLSSPVTKSFNRGEC

SEQ ID NO: 7 - protein, 447 aa, Artificial Sequence
  Synthetic construct
QVQLVESGGGVVQPGRSLRLSCAASGFTFSSYTMHWVRQAPGKGLEWVTFISYDGNNKYYADSVKGRFTISRDNSKNTLYLQMNSLRAEDTAIYYCARTGWLGPFDYWGQGTLVTVSSASTKGPSVFPLAPSSKSTSGGTAALGCLVKDYFPEPVTVSWNSGALTSGVHTFPAVLQSSGLYSLSSVVTVPSSSLGTQTYICNVNHKPSNTKVDKRVEPKSCDKTHTCPPCPAPELLGGPSVFLFPPKPKDTLMISRTPEVTCVVVDVSHEDPEVKFNWYVDGVEVHNAKTKPREEQYNSTYRVVSVLTVLHQDWLNGKEYKCKVSNKALPAPIEKTISKAKGQPREPQVYTLPPSRDELTKNQVSLTCLVKGFYPSDIAVEWESNGQPENNYKTTPPVLDSDGSFFLYSKLTVDKSRWQQGNVFSCSVMHEALHNHYTQKSLSLSPG

SEQ ID NO: 8 - protein, 215 aa, Artificial Sequence
  Synthetic construct
EIVLTQSPGTLSLSPGERATLSCRASQSVGSSYLAWYQQKPGQAPRLLIYGAFSRATGIPDRFSGSGSGTDFTLTISRLEPEDFAVYYCQQYGSSPWTFGQGTKVEIKRTVAAPSVFIFPPSDEQLKSGTASVVCLLNNFYPREAKVQWKVDNALQSGNSQESVTEQDSKDSTYSLSSTLTLSKADYEKHKVYACEVTHQGLSSPVTKSFNRGEC

SEQ ID NO: 9 - protein, 205 aa, Artificial Sequence
  Synthetic construct
ACPWAVSGARASPGSAASPRLREGPELSPDDPAGLLDLRQGMFAQLVAQNVLLIDGPLSWYSDPGLAGVSLTGGLSYKEDTKELVVAKAGVYYVFFQLELRRVVAGEGSGSVSLALHLQPLRSAAGAAALALTVDLPPASSEARNSAFGFQGRLLHLSAGQRLGVHLHTEARARHAWQLTQGATVLGLFRVTPEIPAGLPSPRSE

SEQ ID NO: 10 - protein, 150 aa, Artificial Sequence [sequence omitted]

SEQ ID NO: 11 - protein, 7 aa, Artificial Sequence
  Synthetic construct
EPKSCDK

SEQ ID NO: 12 - DNA, 1032 bp, Artificial Sequence
  Synthetic construct
gctagcaccaagggcccctccgtgttccctctggccccctccagcaagtccacctctggcggcaccgccgctctgggctgcctggtcaaggactacttccccgagcccgtgaccgtgtcctggaactctggcgctctgacctccggcgtgcacaccttccctgccgtgctgcagtcctccggcctgtactccctgtcctccgtcgtgaccgtgccctccagctctctgggcacccagacctacatctgcaacgtgaaccacaagccctccaacaccaaggtggacaagaaggtggaacccaagtcctgcgacaagacccacacctgtcccccctgccctgcccctgagctcctgggaggccctagcgtgttcctgttccccccaaagcccaaggacaccctgatgatctcccggacccccgaagtgacctgcgtggtggtggacgtgtcccacgaggaccctgaagtgaagttcaattggtacgtggacggcgtggaagtgcacaacgccaagaccaagcccagagaggaacagtacaactccacctaccgggtggtgtccgtgctgaccgtgctgcaccaggactggctgaacggcaaagagtacaagtgcaaggtgtccaacaaggccctgcctgcccccatcgaaaagaccatctccaaggccaagggccagccccgcgagcctcaggtgtacaccctgccccctagccgggaagagatgaccaagaaccaggtgtccctgacctgtctggtcaagggcttctacccctccgatatcgccgtggaatgggagtccaacggccagcccgagaacaactacaagaccaccccccctgtgctggactccgacggctcattcttcctgtactccaagctgaccgtggacaagtcccggtggcagcagggcaacgtgttctcctgctccgtgatgcacgaggccctgcacaaccactacacccagaagtccctgtccctgagcccaggcaaaggcggaggcggatctggcggcggaggatctggtggcggatcc

SEQ ID NO: 13 - DNA, 425 bp, Artificial Sequence
  Synthetic construct
ggatccaccatccccccacacgtgcagaaatccgtgaacaacgacatgatcgtgaccgacaacaacggcgctgtgaagttcccccagctgtgcaagttctgcgacgtgcggttctctacctgcgacaaccagaaatcctgcatgtccaactgctccatcacctccatctgcgagaagccccaggaagtgtgcgtcgccgtctggcggaagaacgacgagaacatcaccctggaaaccgtgtgccacgaccccaagctgccctaccacgacttcatcctggaagatgccgcctcccccaagtgcatcatgaaggaaaagaagaagcccggcgagactttcttcatgtgcagctgctcctccgacgagtgcaacgacaacatcatcttctccgaagagtacaacacctccaaccccgactgaagctt

SEQ ID NO: 14 - DNA, 430 bp, Artificial Sequence
  Synthetic construct
gcggccgccatgaacttcggcctgcggctgatcttcctggtgctgaccctgaagggcgtgcagtgcgaggtgcagctggtggaatccggcggaggcctggtccagcctggcggatctctgagactgtcctgcgccgcctccggcttcaacatcaaggacacctacatccactgggtccgacaggcccctggcaagggcctggaatgggtggcccggatctaccccaccaacggctacaccagatacgccgactccgtgaagggccggttcaccatctccgccgacacctccaagaacaccgcctacctgcagatgaactccctgcgggccgaggacaccgccgtgtactactgctccagatggggaggcgacggcttctacgccatggactactggggccagggcaccctggtcaccgtgctccgctagc

SEQ ID NO: 15 - DNA, 442 bp, Artificial Sequence
  Synthetic construct
gcggccgccatggaatcccagacccaggtgctgatctccctgctgttctgggtgtccggcacctgtggcgacatccagatgacccagtccccctccagcctgtccgcctctgtgggcgacagagtgaccatcacctgtcgggcctcccaggacgtgaacaccgccgtggcctggtatcagcagaagcccggcaaggcccccaagctgctgatctactccgcctccttcctgtactccggcgtgccctcccggttctccggctctagatccggcaccgactttaccctgaccatctccagcctgcagcccgaggacttcgccacctactactgccagcagcactacaccaccccccccacctttggccagggcaccaaggtggaaatcaagcggaccgtggccgctccctccgtgttcatccccaccctccgacgagcagctg

SEQ ID NO: 16 - DNA, 1032 bp, Artificial Sequence
  Synthetic construct
gctagcaccaagggcccctccgtgtttcccctggccccctccagcaagtccacctctggcggcaccgccgctctgggctgcctggtcaaggactacttccccgagcccgtgaccgtgtcctggaactctggcgctctgacctccggcgtgcacaccttccctgccgtgctgcagtcctccggcctgtactccctgtcctccgtcgtgaccgtgccctccagctctctgggcacccagacctacatctgcaacgtgaaccacaagccctccaacaccaaggtggacaagcgggtggaacccaagtcctgcgacaagacccacacctgtcccccctgccctgcccctgaactgctgggaggcccttccgtgttcctgttccccccaaagcccaaggacaccctgatgatctcccggacccccgaagtgacctgcgtggtggtggacgtgtcccacgaggaccctgaagtgaagttcaattggtacgtggacggcgtggaagtgcacaacgccaagaccaagcccagagaggaacagtacaactccacctaccgggtggtgtccgtgctgaccgtgctgcaccaggactggctgaacggcaaagagtacaagtgcaaggtgtccaacaaggccctgcctgcccccatcgaaaagaccatctccaaggccaagggccagccccgcgagcctcaggtgtacaccctgcctcccagccgggacgagctgaccaagaaccaggtgtccctgacctgtctggtcaagggcttctacccctccgatatcgccgtggaatgggagtccaacggccagcccgagaacaactacaagaccaccccccctgtgctggactccgacggctcattcttcctgtactccaagctgaccgtggacaagtcccggtggcagcagggcaacgtgttctcctgctccgtgatgcacgaggccctgcacaaccactacacccagaagtccctgtctctgagccccggcaaaggcggcggaggatctggcggtggcggatcaggcggaggatcc

SEQ ID NO: 17 - DNA, 427 bp, Artificial Sequence
  Synthetic construct
gcggccgccatgaacttcggcctgcggctgatcttcctggtgctgaccctgaagggcgtgcagtgccaggtgcagctgaagcagtccggacctggcctggtgcagccttcccagtccctgtccatcacctgtaccgtgtccggcttctccctgaccaactacggcgtgcactgggtccgacagtccccaggcaagggcctggaatggctgggagtgatttggagcggcggcaacaccgactacaacacccccttcacctcccggctgtccatcaacaaggacaactccaagtcccaggtgttcttcaagatgaactccctgcagtccaacgacaccgccatctactactgcgccagagccctgacctactatgactacgagttcgcctactggggacagggcaccctggtcaccgtgtctcgctagc

SEQ ID NO: 18 - DNA, 442 bp, Artificial Sequence
  Synthetic construct
gcggccgccatggaatcccagacccaggtgctgatctccctgctgttctgggtgtccggcacctgtggcgacatcctgctgacccagtcccccgtgatcctgtccgtgtctcctggcgagcgggtgtccttctcctgccgggcctcccagtccatcggcaccaacatccactggtatcagcagcggaccaacggctcccctcggctgctgattaagtacgcctccgagtctatctccggcatcccctcccggttctccggctctggctccggcaccgacttcaccctgtccatcaactccgtggaatccgaggatatcgccgactactactgccagcagaacaacaactggcccaccaccttcggcgctggcaccaagctggaactgaagcggaccgtggccgctccctccgtgttcatccccaccctccgacgagcagctg

SEQ ID NO: 19 - DNA, 424 bp, Artificial Sequence
  Synthetic construct
gcggccgccatgaacttcggcctgcggctgatcttcctggtgctgaccctgaagggcgtgcagtgccaggtgcagctggtggaatccggcggaggcgtggtgcagcctggcagatccctgagactgtcctgcgccgcctccggcttcaccttctccagctacaccatgcactgggtccgacaggcccctggcaagggcctggaatgggtcaccttcatcagctacgacggcaacaacaagtactacgccgactccgtgaagggccggttcaccatctcccgggacaactccaagaacaccctgtacctgcagatgaactccctgcgggccgaggacaccgccatctactactgcgcccggaccggctggctgggcccttttgattactggggccagggcaccctggtcaccgtgtcctcctagc

SEQ ID NO: 20 - DNA, 445 bp, Artificial Sequence
  Synthetic construct
gcggccgccatggaatcccagacccaggtgctgatctccctgctgttctgggtgtccggcacctgtggcgagatcgtgctgacccagtcccccggcaccctgtctctgagccctggcgagagagccaccctgtcctgcagagcctcccagtccgtgggctcctcctacctggcttggtatcagcagaagcccggccaggcccctcggctgctgatctacggcgctttctctcgggccaccggcatccctgaccggttctctggctccggctccggcaccgacttcaccctgaccatctcccggctggaacccgaggacttcgccgtgtactactgccagcagtacggctcctccccctggacctttggccagggcaccaaggtggaaatcaagcggaccgtggccgctccctccgtgttccttcccaccctccgacgagcagctg

SEQ ID NO: 21 - DNA, 1035 bp, Artificial Sequence
  Synthetic construct
gctagcacaaagggccctagtgtgtttcctctggctccctcttccaaatccacttctggtggcactgctgctctgggatgcctggtgaaggattactttcctgaacctgtgactgtctcatggaactctggtgctctgacttctggtgtccacactttccctgctgtgctgcagtctagtggactgtactctctgtcatctgtggtcactgtgccctcttcatctctgggaacccagacctacatttgtaatgtgaaccacaaaccatccaacactaaagtggacaaaaaagccgaacccaaatcctgtgacaaaacccacacctgcccaccttgtcctgcccctgaactgctgggaggaccttctgtgtttctgttcccaccaaaaccaaaagataccctgatgatctctagaacccctgaggtgacatgtgtggtggtggatgtgtctcatgaggaccctgaggtcaaatttaattggtacgtcgatggagtggaagtccacaatgccaaaaccaagcctagagaggaacagtacaattcaacctacagagtcgtcagtgtgctgactgtgctgcatcaggattggctgaatggcaaggaatacaagtgtaaagtctcaaacaaggccctgcctgctccaattgagaaaacaatctcaaaggccaagggacagcctagggaaccccaggtctacaccctgccaccttcacgcgacgaactgaccaaaaaccaggtgtccctgacatgcctggtcaaaggcttctacccttctgacattgctgtggagtgggagtcaaatggacagcctgagaacaactacaaaacaaccccccctgtgctggattctgatggctctttctttctgtactccaaactgactgtggacaagtctagatggcagcaggggaatgtcttttcttgctctgtcatgcatgaggctctgcataaccactacactcagaaatccctgtctctgtctcccgggaaaggcggcggaggatctggcggaggcggttctggtggtggcggatcc

SEQ ID NO: 22 - DNA, 435 bp, Artificial Sequence
  Synthetic construct
gcggccgccatgaattttggactgaggctgattttcctggtgctgaccctgaaaggcgtccagtgtcaggtgcagctgcagcagcctggtgccgagctcgtgaaacctggcgcctccgtgaagatgtcctgcaaggcctccggctacaccttcaccagctacaacatgcactgggtcaagcagacccccggcagaggcctggaatggatcggcgctatctaccccggcaacggcgacacctcctacaaccagaagttcaagggcaaggccaccctgaccgccgacaagtcctcttccaccgcctacatgcagctgtcctccctgacctccgaggactccgccgtgtactactgcgcccggtctacctactacggcggcgactggtacttcaacgtgtggggcgctggcaccaccgtgaccgtgtctgctgctagc

SEQ ID NO: 23 - DNA, 405 bp, Artificial Sequence
  Synthetic construct
gcggccgccatgaattttggactgaggctgattttcctggtgctgaccctgaaaggcgtccagtgtcagatcgtgctgtcccagtcccctgccatcctgtctgctagccctggcgagaaagtgacaatgacctgccgggcctcctcctccgtgtcctacatccactggttccagcagaagcccggctccagccccaagccttggatctacgccacctccaacctggcctctggcgtgccagtgcggttttccggctctggctctggcacctcctactccctgaccatctctcgggtggaagccgaggatgccgccacctactactgccagcagtggaccagcaacccccccacatttggcggaggcaccaagctggaaatcaagcggaccgtggcggcgccctct

SEQ ID NO: 24 - DNA, 631 bp, Artificial Sequence
  Synthetic construct
ggatccgcctgtccttgggccgtgtccggcgctagagcctctcctggctctgccgcctcccccagactgagagagggccctgagctgtcccctgacgatcctgccggcctgctggacctgagacagggcatgtttgcccagctggtggcccagaacgtgctgctgatcgacggccccctgtcctggtactctgatcctggcctggccggcgtgtccctgaccggcggactgtcctacaaagaggacaccaaagaactggtggtggccaaggctggcgtgtactacgtgttctttcagctggaactgcggcgggtggtggccggcgagggctctggatctgtgtccctggccctgcatctgcagcccctgagatctgccgctggcgccgctgctctggccctgacagtggatctgcctcctgcctcctccgaggcccggaactccgcattcgggtttcagggccggctgctgcacctgtctgctggccagagactgggagtgcatctgcacaccgaggccagagccagacacgcctggcagctgacccagggcgctaccgtgctgggcctgttcagagtgacccccgagatcccagccggcctgcccagccctagatccgagtgataagctt

SEQ ID NO: 25 - DNA, 1458 bp, Artificial Sequence
  Synthetic construct
gcggccgccatgaattttggactgaggctgattttcctggtgctgaccctgaaaggcgtccagtgtcaggtgcagctgcaggaatctggccctggactcgtgcggccttcccaaaccctgtctctgacctgtaccgtgtccggctactccatcacctccgaccacgcctggtcttgggtgcgacagcctcctggcagaggcctggaatggatcggctacatctcctactccggcatcaccacctacaaccccagcctgaagtccagagtgaccatgctgcgggacacctccaagaaccagttctccctgcggctgtcctccgtgaccgctgctgataccgccgtgtactactgcgccagatctctggccaggaccaccgccatggattactggggccagggctccctcgtgaccgtgtcctctgctagcaccaagggcccctccgtgttccctctggccccttcctctaaatctacctctggcggcaccgccgctctgggctgcctcgtgaaggactacttccccgagcccgtgacagtgtcttggaactctggcgccctgacctccggcgtgcacacctttccagctgtgctgcagtcctccggcctgtactccctgtccagcgtcgtgactgtgccctcctcatctctgggcacccagacctacatctgcaacgtgaaccacaagccctccaacaccaaggtggacaagaaggtggaacccaagtcctgcgacaagacccacacctgtcccccttgtcctgcccctgaactgctgggcggaccctctgtgttcctgttcccaccaaaaccgaaagacaccctgatgatctcccggacccccgaagtgacctgcgtggtggtggatgtgtcccacgaggaccctgaagtgaagttcaattggtacgtggacggcgtggaagtgcacaacgccaagaccaagcctagagaggaacagtacaactccacctaccgggtggtgtccgtgctgaccgtgctgcaccaggattggctgaacggcaaagagtacaagtgcaaggtgtccaacaaggccctgcctgcccccatcgaaaagaccatctccaaggccaagggccagccacgggaaccccaggtgtacacactgccccctagccgcgacgagctgaccaagaatcaggtgtccctgacatgcctcgtgaaaggcttctacccctccgatatcgccgtggaatgggagtccaacggccagcctgagaacaactacaagaccaccccccctgtgctggactccgacggctcattcttcctgtactcaaagctgacagtggacaagtcccggtggcagcagggcaacgtgttctcctgctccgtgatgcacgaggccctgcacaaccactacacccagaagtccctgtccctgagccccgggaaaggcggcggaggatctggcggaggcggttctggtggtggcggatcc

SEQ ID NO: 26 - DNA, 405 bp, Artificial Sequence
  Synthetic construct
gcggccgccatgaattttggactgaggctgattttcctggtgctgaccctgaaaggcgtccagtgtgacatccagatgacccagtccccctccagcctgtctgcctctgtgggcgacagagtgaccatcacctgtcgggcctcccaggacatctcctcctacctgaactggtatcagcagaagcccggcaaggcccccaagctgctgatctactacacctcccggctgcactccggcgtgccctctagattttccggctctggctccggcaccgactttaccttcaccatcagctccctgcagcccgaggatatcgccacctactactgccagcaaggcaacaccctgccctacacctttggccagggcaccaaggtggaaatcaagcggaccgtggcggcgccc

SEQ ID NO: 27 - DNA, 1455 bp, Artificial Sequence
  Synthetic construct
gcggccgccatgaattttggactgaggctgattttcctggtgctgaccctgaaaggcgtccagtgtcaggtgcagctgcagcagtggggagctggactgctgaagccctccgagacactgtctctgacctgcgctgtgtacggcggctccttctccggctactactggtcctggattcggcagtcccctgagaagggcctggaatggatcggcgagatcaaccacggcggctacgtgacctacaaccccagcctggaatccagagtgaccatctccgtggacacctccaagaaccagttctccctgaagctgtcctccgtgaccgccgctgataccgccgtgtactactgcgccagagactacggccctggcaactacgactggtacttcgacctgtggggcagaggcaccctcgtgaccgtgtcctctgctagcaccaagggcccctccgtgtttcctctggccccttgctcacgctccacctccgaatctaccgccgctctgggctgcctcgtgaaggactacttccccgagcccgtgactgtgtcttggaactctggcgccctgacctccggcgtgcacacctttccagctgtgctgcagtcctccggcctgtactccctgtccagcgtcgtgacagtgccctccagctctctgggcaccaagacctacacctgtaacgtggaccacaagccctccaacaccaaggtggacaagcgggtggaatctaaatacggccctccctgccctccttgcccagcccctgaatttctgggcggaccttccgtgttcctgttccccccaaaacccaaggacaccctgatgatctcccggacccccgaagtgacctgcgtggtggtggatgtgtcccaggaagatcccgaggtgcagttcaattggtacgtggacggcgtggaagtgcacaacgccaagaccaagcctagagaggaacagttcaactccacctaccgggtggtgtccgtgctgaccgtgctgcaccaggattggctgaacggcaaagagtacaagtgcaaggtgtccaacaagggcctgcccagctccatcgaaaagaccatcagcaaggccaagggccagccccgggaaccccaggtgtacacactgcctccaagccaggaagagatgaccaagaatcaggtgtccctgacctgtctcgtgaaaggcttctacccctccgatatcgccgtggaatgggagtccaacggccagcctgagaacaactacaagaccaccccccctgtgctggactccgacggcagcttcttcctgtactctcgcctgaccgtggacaagtcccggtggcaggaaggcaacgtgttctcctgctccgtgatgcacgaggccctgcacaaccactacacccagaagtccctgtccctgtctctggggaaaggcggcggaggatctggcggaggcggttctggtggtggcggatcc

SEQ ID NO: 28 - DNA, 411 bp, Artificial Sequence
  Synthetic construct
gcggccgccatgaattttggactgaggctgattttcctggtgctgaccctgaaaggcgtccagtgtgagatcgtgctgacccagtctcctgccaccctgtctctgagccctggcgagagagctaccctgtcctgccgtgcctcccaatccgtgtcctcttacctggcctggtatcagcaaaagcccggccaggctccccggctgctgatctacgatgcctccaatagagccaccggcatccctgccagattctccggctctggctctggcaccgactttaccctgaccatctcctctctggaacccgaggacttcgccgtgtactactgccagcagcggtccaactggcctcccgccctgacatttggcggaggcaccaaggtggaaatcaagcggaccgtggcggcgccc

SEQ ID NO: 29 - protein, 449 aa, Artificial Sequence
  Synthetic construct
QVQLVQSGAEVKKPGETVKISCKASDYTFTYYGMNWVKQAPGQGLKWMGWIDTTTGEPTYAQKFQGRIAFSLETSASTAYLQIKSLKSEDTATYFCARRGPYNWYFDVWGQGTTVTVSSASTKGPSVFPLAPSSKSTSGGTAALGCLVKDYFPEPVTVSWNSGALTSGVHTFPAVLQSSGLYSLSSVVTVPSSSLGTQTYICNVNHKPSNTKVDKKVEPKSCDKTHTCPPCPAPELLGGPSVFLFPPKPKDTLMISRTPEVTCVVVDVSHEDPEVKFNWYVDGVEVHNAKTKPREEQYNSTYRVVSVLTVLHQDWLNGKEYKCKVSNKALPAPIEKTISKAKGQPREPQVYTLPPSRDELTKNQVSLTCLVKGFYPSDIAVEWESNGQPENNYKTTPPVLDSDGSFFLYSKLTVDKSRWQQGNVFSCSVMHEALHNHYTQKSLSLSPGK

SEQ ID NO: 30 - protein, 219 aa, Artificial Sequence
  Synthetic construct
DIVMTQSPLSVPVTPGEPVSISCRSSKSLLHSNGNTYLYWFLQRPGQSPQLLIYRMSNLVSGVPDRFSGSGSGTAFTLRISRVEAEDVGVYYCLQHLEYPFTFGPGTKLELKRTVAAPSVFIFPPSDEQLKSGTASVVCLLNNFYPREAKVQWKVDNALQSGNSQESVTEQDSKDSTYSLSSTLTLSKADYEKHKVYACEVTHQGLSSPVTKSFNRGEC

SEQ ID NO: 31 - protein, 460 aa, Artificial Sequence
  Synthetic construct
EVQLVQSGAEVKKPGSSVKVSCKASGGTFSSYAISWVRQAPGQGLEWMGGIIPIFGTANYAQKFQGRVTITADKSTSTAYMELSSLRSEDTAVYYCARAPLRFLEWSTQDHYYYYYMDVWGKGTTVTVSSASTKGPSVFPLAPSSKSTSGGTAALGCLVKDYFPEPVTVSWNSGALTSGVHTFPAVLQSSGLYSLSSVVTVPSSSLGTQTYICNVNHKPSNTKVDKKVEPKSCDKTHTCPPCPAPELLGGPSVFLFPPKPKDTLMISRTPEVTCVVVDVSHEDPEVKFNWYVDGVEVHNAKTKPREEQYNSTYRVVSVLTVLHQDWLNGKEYKCKVSNKALPAPIEKTISKAKGQPREPQVYTLPPSREEMTKNQVSLTCLVKGFYPSDIAVEWESNGQPENNYKTTPPVLDSDGSFFLYSKLTVDKSRWQQGNVFSCSVMHEALHNHYTQKSLSLSPGK

SEQ ID NO: 32 - protein, 213 aa, Artificial Sequence
  Synthetic construct
SSELTQDPAVSVALGQTVRITCQGDSLRSYYATWYQQKPGQAPILVIYGENKRPSGIPDRFSGSSSGNTASLTITGAQAEDEADYYCKSRDGSGQHLVFGGGTKLTVLGQPKAAPSVTLFPPSSEELQANKATLVCLISDFYPGAVTVAWKADSSPVKAGVETTTPSKQSNNKYAASSYLSLTPEQWKSHRSYSCQVTHEGSTVEKTVAPAEC

SEQ ID NO: 33 - protein, 449 aa, Artificial Sequence
  Synthetic construct
QVQLQQSGAEVKKFGASVKVSCEASGYTFPSYVLHWVKQAPGQGLEWIGYINPYNDGTQTNKKFKGKATLTRDTSINTAYMELSRLRSDDTAVYYCARGFGGSYGFAYNGQGTLVTVSSASTKGPSVFPLAPSSKSTSGGTAALGCLVKDYFPEPVTVSWNSGALTSGVNTFPAVLQSSGLYSLSSVVTVPSSSLGTQTYICNVNHKPSNTKVDKRVEPKSCDKTHTCPPCPAPELLGGPSVFLFPPKPKDTLNISRTPEVTCVVVDVSHEDPEVKFNWYVDGVEVHNAKTKPREEQYNSTYRVVSVLTVLHQDWLNGKEYKCKVSNKALPAPIEKTISKAKGQPREPQVYTLPPSREEMTKNQVSLTCLVKGFYPSDIAVEWESNGQPENNYKTTPPVLDSDGSFFLYSKLTVDKSRWQQGNVFSCSVNHEALHNHYTQKSLSLSPGK

SEQ ID NO: 34 - protein, 215 aa, Artificial Sequence
  Synthetic construct
DIQLTQSPSSLSASVGDRVTMTCSASSSVSSSYLYWYQQKPGKAPKLWIYSTSNLASGVPARFSGSGSGTDFTLTISSLQPEDSASYFCHQWNRYPYTFGGGTRLEIKRTVAAPSVFIFPPSDEQLKSGTASVVCLLNNFYEAKVQWKVDNALQSGNSQESVTEQDSKDSTYSLSSTLTLSPRKADYEKHKVYACEVTHQGLSSPVTKSFNRGEC

SEQ ID NO: 35 - protein, 450 aa, Artificial Sequence
  Synthetic construct
EVQLLESGGDLVQPGGSLRLSCAASGFTFSNYAMSWVRQAPGKGLEWVSAITPSGGSTNYADSVKGRFTISRDNSQNTLYLQMNSLRVEDTAVYICGRVPYRSTWYPLYWGQGTLVTVSSASTKGPSVFPLAPSSKSTSGGTAALGCLVKDYFPEPVTVSWNSGALTSGVHTFPAVLQSSGLYSLSSVVTVPSSSLGTQTYICNVNHKPSNTKVDKKVEPKSCDKTHTCPPCPAPELLGGPSVFLFPPKPKDTLMISRTPEVTCVVVDVSHEDPEVKFNWYVDGVEVHNAKTKPREEQYNSTYRVVSVLTVLHQDWLNGKEYKCKVSNKALPAPIEKTISKAKGQPREPQVYTLPPSRDELTKNQVSLTCLVKGFYPSDIAVEWESNGQPENNYKTTPPVLDSDGSFFLYSKLTVDKSRWQQGNVFSCSVMHEALHNHYTQKSLSLSPGK

SEQ ID NO: 36 - protein, 214 aa, Artificial Sequence
  Synthetic construct
DIQMTQSPSSLSASVGDRVTITCRASQDISNYLAWFQQKPGKAPKSLIYAASSLHSKVPTQFSGSGSGTDFTLTISSLQPEDFATYYCLQYSTYPITFGGGTKVEIKRTVAAPSVFIFPPSDEQLKSGTASVVCLLNNFYPREAKVQWKVDNALQSGNSQESVTEQDSKDSTYSLSSTLTLSKADYEKHKVYACEVTHQGLSSPVTKSFNRGEC